European Patent Specification EP 4 139 286 B1, published February 26, 2025. Title: SUBSTITUTED AMINOTHIAZOLES AS DGKZETA INHIBITORS FOR IMMUNE ACTIVATION. Applicant: Bayer AG Deutsches Krebsforschungszentrum (DKFZ). The sequence listing filed with the application follows.

SEQUENCE LISTING (5 sequences)

SEQ ID NO: 1 - protein, 938 aa, human DGKzM1
  DGKz hu 1 encoding human DGKzM1 to V928 plus N-terminal Flag-Tag
MGDYKDDDDKMEPRDGSPEARSSDSESASASSSGSERDAGPEPDKAPRRLNKRRFPGLRLFGHRKAITKSGLQHLAPPPPTPGAPCSESERQIRSTVDWSESATYGEHIWFETNVSGDFCYVGEQYCVARMLKSVSRRKCAACKIVVHTPCIEQLEKINFRCKPSFRESGSRNVREPTFVRHHWVHRRRQDGKCRHCGKGFQQKFTFHSKEIVAISCSWCKQAYHSKVSCFMLQQIEEPCSLGVHAAVVIPPTWILRARRPQNTLKASKKKKRASFKRKSSKKGPEEGRWRPFIIRPTPSPLMKPLLVFVNPKSGGNQGAKIIQSFLWYLNPRQVFDLSQGGPKEALEMYRKVHNLRILACGGDGTVGWILSTLDQLRLKPPPPVAILPLGTGNDLARTLNWGGGYTDEPVSKILSHVEEGNVVQLDRWDLHAEPNPEAGPEDRDEGATDRLPLDVFNNYFSLGFDAHVTLEFHESREANPEKFNSRFRNKMFYAGTAFSDFLMGSSKDLAKHIRVVCDGMDLTPKIQDLKPQCVVFLNIPRYCAGTMPWGHPGEHHDFEPQRHDDGYLEVIGFTMTSLAALQVGGHGERLTQCREVVLTTSKAIPVQVDGEPCKLAASRIRIALRNQATMVQKAKRRSAAPLHSDQQPVPEQLRIQVSRVSMHDYEALHYDKEQLKEASVPLGTVVVPGDSDLELCRAHIERLQQEPDGAGAKSPTCQKLSPKWCFLDATTASRFYRIDRAQEHLNYVTEIAQDEIYILDPELLGASARPDLPTPTSPLPTSPCSPTPRSLQGDAAPPQGEELIEAAKRNDFCKLQELHRAGGDLMHRDEQSRTLLHHAVSTGSKDVVRYLLDHAPPEILDAVEENGETCLHQAAALGQRTICHYIVEAGASLMKTDQQGDTPRQRAEKAQDTELAAYLENRQHYQMIQREDQETAV

SEQ ID NO: 2 - protein, 8 aa, mouse
  SIINFEKL
SIINFEKL

SEQ ID NO: 3 - protein, 30 aa, chicken
  Ovalbumin antigen OVA-30
SMLVLLPDEVSGLEQLESIINFEKLTEWTS

SEQ ID NO: 4 - protein, 8 aa, synthetic organisms
  FLAG-Tag
DYKDDDDK

SEQ ID NO: 5 - protein, 6 aa, synthetic organisms
  Kozak sequence for translation initiation
GCCACC